European Patent Specification EP 3 908 585 B1, published March 6, 2024. Title: IL-17 RECEPTOR MODULATORS. Applicant: Eli Lilly and Company. The sequence listing filed with the application follows.

SEQUENCE LISTING (3 sequences)

SEQ ID NO: 1 - protein, 176 aa, Artificial sequence
  Synthetic construct
MTPGKTSLVSLLLLLSLEAIVKAGITIPRNPGCPNSEDKNFPRTVMVNLNIHNRNTNTNPKRSSDYYNRSTSPWNLHRNEDPERYPSVIWEAKCRHLGCINADGNVDYHMNSVPIQQEILVLRREPPHCPNSFRLEKILVSVGCTCVTPIVHHVAGLNDIFEAQKIEWHEHHHHHH

SEQ ID NO: 2 - protein, 323 aa, Artificial sequence
  Synthetic construct
MALKDNTVPLKLIALLANGEFHSGEQLGETLGMSRAAINKHIQTLRDWGVDVFTVPGKGYSLPEPIQLLNAKQILGQLDGGSVAVLPVIDSTNQYLLDRIGELKSGDACIAEYQQAGRGRRGRKWFSPFGANLYLSMFWRLEQGPAAAIGLSLVIGIVMAEVLRKLGADKVRVKWPNDLYLQDRKLAGILVELTGKTGDAAQIVIGAGINMAMRRVEESVVNQGWITLQEAGINLDRNTLAAMLIRELRAALELFEQEGLAPYLSRWEKLDNFINRPVKLIIGDKEIFGISRGIDKQGALLLEQDGIIKPWMGGEISLRSAEK

SEQ ID NO: 3 - protein, 331 aa, Artificial sequence
  Synthetic construct
MGAARSPPSAVPGPLLGLLLLLLGVLAPGGASLRLLDHRALVCSQPGLNCTVKNSTCLDDSWIHPRNLTPSSPKDLQIQLHFAHTQQGDLFPVAHIEWTLQTDASILYLEGAELSVLQLNTNERLCVRFEFLSKLRHHHRRWRFTFSHFVVDPDQEYEVTVHHLPKPIPDGDPNHQSKNFLVPDCEHARMKVTTPCMSSGSLWDPDITVETLEAHQLRVSFTLWNESTHYQILLTSFPHMENHSCFEHMHHIPAPRPEEFHQRSDVTLTLRNLKGCCRHQVQIQPFFSSCLNDCLRHSATVSCPEMPDTPEPIPDYMLVPRGSDYKDDDDK